European Patent Specification EP 3 365 437 B1, published June 4, 2025. Title: METHODS AND PRODUCTS FOR GENETIC ENGINEERING. Applicant: INSTITUT NATIONAL DE LA SANTE ET DE LA RECHERCHE MEDICALE (INSERM) CENTRE NATIONAL DE LA RECHERCHE SCIENTIFIQUE (CNRS) ECOLE NORMALE SUPERIEURE DE LYON UNIVERSITE CLAUDE BERNARD LYON 1. The sequence listing filed with the application follows.

SEQUENCE LISTING (40 sequences)

SEQ ID NO: 1 - DNA, 25 bp, Artificial Sequence
  YFPgRNA1f primer
  YFPgRNA1f primer
caccgcgaggagctgttcaccgggg

SEQ ID NO: 2 - DNA, 25 bp, Artificial Sequence
  YFPgRNA1r primer
  YFPgRNA1r primer
aaacccccggtgaacagctcctcgc

SEQ ID NO: 3 - DNA, 25 bp, Artificial Sequence
  YFPgRNA2f primer
  YFPgRNA2f primer
caccgtcaccataccggtagccagc

SEQ ID NO: 4 - DNA, 25 bp, Artificial Sequence
  YFPgRNA2r primer
  YFPgRNA2r primer
aaacgctggctaccggtatggtgac

SEQ ID NO: 5 - DNA, 25 bp, Artificial Sequence
  hMyd88gRNA1f primer
  hMyd88gRNA1f primer
caccggagacctcaagggtagaggt

SEQ ID NO: 6 - DNA, 25 bp, Artificial Sequence
  hMyd88gRNA1r primer
  hMyd88gRNA1r primer
aaacacctctacccttgaggtctcc

SEQ ID NO: 7 - DNA, 25 bp, Artificial Sequence
  hMyd88gRNA2f primer
  hMyd88gRNA2f primer
caccggcagccatggcgggcggtcc

SEQ ID NO: 8 - DNA, 25 bp, Artificial Sequence
  hMyd88gRNA2r primer
  hMyd88gRNA2r primer
aaacggaccgcccgccatggctgcc

SEQ ID NO: 9 - DNA, 25 bp, Artificial Sequence
  mMyd88gRNA1f primer
  mMyd88gRNA1f primer
caccggagcgtactggacggcaccg

SEQ ID NO: 10 - DNA, 25 bp, Artificial Sequence
  mMyd88gRNA1r primer
  mMyd88gRNA1r primer
aaaccggtgccgtccagtacgctcc

SEQ ID NO: 11 - DNA, 25 bp, Artificial Sequence
  mMyd88gRNA2f primer
  mMyd88gRNA2f primer
caccggcccatctcctccgccagca

SEQ ID NO: 12 - DNA, 25 bp, Artificial Sequence
  mMyd88gRNA2r primer
  mMyd88gRNA2r primer
aaactgctggcggaggagatgggcc

SEQ ID NO: 13 - DNA, 25 bp, Artificial Sequence
  DDX3gRNA1f primer
  DDX3gRNA1f primer
caccgagggatgagtcatgtggcag

SEQ ID NO: 14 - DNA, 25 bp, Artificial Sequence
  DDX3gRNA1r primer
  DDX3gRNA1r primer
aaacctgccacatgactcatccctc

SEQ ID NO: 15 - DNA, 51 bp, Artificial Sequence
  YFPf primer
  YFPf primer
tctaatacgactcactatagggagaggtctatataagcagagctcgtttag

SEQ ID NO: 16 - DNA, 25 bp, Artificial Sequence
  YFPr primer
  YFPr primer
ggccatgatatagacgttgtggctg

SEQ ID NO: 17 - DNA, 23 bp, Artificial Sequence
  hMyd88f2 primer
  hMyd88f2 primer
ttacgccccccacatcacccgcc

SEQ ID NO: 18 - DNA, 24 bp, Artificial Sequence
  hMyd88r1 primer
  hMyd88r1 primer
gtctccagttgccggatctccaag

SEQ ID NO: 19 - DNA, 23 bp, Artificial Sequence
  mMyd88f2 primer
  mMyd88f2 primer
ggaaactccacaggcgagcgtac

SEQ ID NO: 20 - DNA, 26 bp, Artificial Sequence
  mMyd88r2 primer
  mMyd88r2 primer
ggcagtcctcctcgatgcgcgacttc

SEQ ID NO: 21 - DNA, 119 bp, Artificial Sequence
  Flag-DDX3 primer
  Flag-DDX3 primer
actcgcttagcagcggaagactccgagttctcggtactcttcagggatggactacaaggacgacgatgacaagagtcatgtggcagtggaaaatgcgctcgggctggaccagcaggtga

SEQ ID NO: 22 - protein, 1958 aa, Artificial Sequence
  GAG-Cas9 fusion protein
  GAG-Cas9 fusion protein
MGQAVTTPLSLTLDHWKDVERTAHNLSVEVRKRRWVTFCSAEWPTFNVGWPRDGTFNPDIITQVKIKVFSPGPHGHPDQVPYIVTWEAIAVDPPPWVRPFVHPKPPLSLPPSAPSLPPEPPLSTPPQSSLYPALTSPLNTKPRPQVLPDSGGPLIDLLTEDPPPYRDPGPPSPDGNGDSGEVAPTEGAPDPSPMVSRLRGRKEPPVADSTTSQAFPLRLGGNGQYQYWPFSSSDLYNWKNNNPSFSEDPAKLTALIESVLLTHQPTWDDCQQLLGTLLTGEEKQRVLLEARKAVRGEDGRPTQLPNDINDAFPLERPDWDYNTQRGRNHLVHYRQLLLAGLQNAGRSPTNLAKVKGITQGPNESPSAFLERLKEAYRRYTPYDPEDPGQETNVAMSFIWQSAPDIGRKLERLEDLKSKTLGDLVREAEKIFNKRETPEEREERIRRETEEKEERRRAEDVQREKERDRRRHREMSKLLATVVSGQRQDRQGGERRRPQLDHDQCAYCKEKGHWARDCPKKPRGPRGPRPQASLLTRSSLYPALTPTGDYKDDDDKMAPKKKRKVGIHGVPAADKKYSIGLDIGTNSVGWAVITDEYKVPSKKFKVLGNTDRHSIKKNLIGALLFDSGETAEATRLKRTARRRYTRRKNRICYLQEIFSNEMAKVDDSFFHRLEESFLVEEDKKHERHPIFGNIVDEVAYHEKYPTIYHLRKKLVDSTDKADLRLIYLALAHMIKFRGHFLIEGDLNPDNSDVDKLFIQLVQTYNQLFEENPINASGVDAKAILSARLSKSRRLENLIAQLPGEKKNGLFGNLIALSLGLTPNFKSNFDLAEDAKLQLSKDTYDDDLDNLLAQIGDQYADLFLAAKNLSDAILLSDILRVNTEITKAPLSASMIKRYDEHHQDLTLLKALVRQQLPEKYKEIFFDQSKNGYAGYIDGGASQEEFYKFIKPILEKMDGTEELLVKLNREDLLRKQRTFDNGSIPHQIHLGELHAILRRQEDFYPFLKDNREKIEKILTFRIPYYVGPLARGNSRFAWMTRKSEETITPWNFEEVVDKGASAQSFIERMTNFDKNLPNEKVLPKHSLLYEYFTVYNELTKVKYVTEGMRKPAFLSGEQKKAIVDLLFKTNRKVTVKQLKEDYFKKIECFDSVEISGVEDRFNASLGTYHDLLKIIKDKDFLDNEENEDILEDIVLTLTLFEDREMIEERLKTYAHLFDDKVMKQLKRRRYTGWGRLSRKLINGIRDKQSGKTILDFLKSDGFANRNFMQLIHDDSLTFKEDIQKAQVSGQGDSLHEHIANLAGSPAIKKGILQTVKVVDELVKVMGRHKPENIVIEMARENQTTQKGQKNSRERMKRIEEGIKELGSQILKEHPVENTQLQNEKLYLYYLQNGRDMYVDQELDINRLSDYDVDHIVPQSFLKDDSIDNKVLTRSDKNRGKSDNVPSEEVVKKMKNYWRQLLNAKLITQRKFDNLTKAERGGLSELDKAGFIKRQLVETRQITKHVAQILDSRMNTKYDENDKLIREVKVITLKSKLVSDFRKDFQFYKVREINNYHHAHDAYLNAVVGTALIKKYPKLESEFVYGDYKVYDVRKMIAKSEQEIGKATAKYFFYSNIMNFFKTEITLANGEIRKRPLIETNGETGEIVWDKGRDFATVRKVLSMPQVNIVKKTEVQTGGFSKESILPKRNSDKLIARKKDWDPKKYGGFDSPTVAYSVLVVAKVEKGKSKKLKSVKELLGITIMERSSFEKNPIDFLEAKGYKEVKKDLIIKLPKYSLFELENGRKRMLASAGELQKGNELALPSKYVNFLYLASHYEKLKGSPEDNEQKQLFVEQHKHYLDEIIEQISEFSKRVILADANLDKVLSAYNKHRDKPIREQAENIIHLFTLTNLGAPAAFKYFDTTIDRKRYTSTKEVLDATLIHQSITGLYETRIDLSQLGGDKRPAATKKAGQAKKKKARA

SEQ ID NO: 23 - protein, 511 aa, Vesicular stomatitis virus
  VSV-G protein
  VSV-G protein
MKCLLYLAFLFIGVNCKFTIVFPHNQKGNWKNVPSNYHYCPSSSDLNWHNDLIGTAIQVKMPKSHKAIQADGWMCHASKWVTTCDFRWYGPKYITQSIRSFTPSVEQCKESIEQTKQGTWLNPGFPPQSCGYATVTDAEAVIVQVTPHHVLVDEYTGEWVDSQFINGKCSNYICPTVHNSTTWHSDYKVKGLCDSNLISMDITFFSEDGELSSLGKEGTGFRSNYFAYETGGKACKMQYCKHWGVRLPSGVWFEMADKDLFAAARFPECPEGSSISAPSQTSVDVSLIQDVERILDYSLCQETWSKIRAGLPISPVDLSYLAPKNPGTGPAFTIINGTLKYFETRYIRVDIAAPILSRMVGMISGTTTERELWDDWAPYEDVEIGPNGVLRTSSGYKFPLYMIGHGMLDSDLHLSSKAQVFEHPHIQDAASQLPDDESLFFGDTGLSKNPIELVEGWFSSWKSSIASFFFIIGLIIGLFLVLRVGIHLCIKLKHTKKRQIYTDIEMNRLGK

SEQ ID NO: 24 - protein, 1742 aa, Artificial Sequence
  GAG PRO POL polyprotein
  GAG PRO POL polyprotein
MGQAVTTPLSLTLDHWKDVERTAHNLSVEVRKRRWVTFCSAEWPTFNVGWPRDGTFNPDIITQVKIKVFSPGPHGHPDQVPYIVTWEAIAVDPPPWVRPFVHPKPPLSLPPSAPSLPPEPPLSTPPQSSLYPALTSPLNTKPRPQVLPDSGGPLIDLLTEDPPPYRDPGPPSPDGNGDSGEVAPTEGAPDPSPMVSRLRGRKEPPVADSTTSQAFPLRLGGNGQYQYWPFSSSDLYNWKNNNPSFSEDPAKLTALIESVLLTHQPTWDDCQQLLGTLLTGEEKQRVLLEARKAVRGEDGRPTQLPNDINDAFPLERPDWDYNTQRGRNHLVHYRQLLLAGLQNAGRSPTNLAKVKGITQGPNESPSAFLERLKEAYRRYTPYDPEDPGQETNVAMSFIWQSAPDIGRKLERLEDLKSKTLGDLVREAEKIFNKRETPEEREERIRRETEEKEERRRAEDVQREKERDRRRHREMSKLLATVVSGQRQDRQGGERRRPQLDHDQCAYCKEKGHWARDCPKKPRGPRGPRPQASLLTLDDTLDDQGGQGQEPPPEPRITLRVGGQPVTFLVDTGAQHSVLTQNPGPLSDKSAWVQGATGGKRYRWTTDRRVHLATGKVTHSFLHVPDCPYPLLGRDLLTKLKAQIHFEGSGAQVVGPMGQPLQVLTLNIEDEYRLHETSKGPDVPLGSTWLSDFPQAWAETGGMGLAVRQAPLIIPLKATSTPVSIKQYPMSQEARLGIKPHIQRLLDQGILVPCQSPWNTPLLPVKKPGTNDYRPVQDLREVNKRVEDIHPTVPNPYNLLSGLPPSHQWYTVLDLKDAFFCLRLHPTSQSLFAFEWRDPEMGISGQLTWTRLPQGFKNSPTLFDEALHRDLADFRIQHPDLILLQYVDDLLLAATSELDCQQGTRALLQTLGDLGYRASAKKAQICQKQVKYLGYLLKEGQRWLTEARKETVMGQPTPKTPRQLREFLGTAGFCRLWIPGFAEMAAPLYPLTKTGTLFEWGPDQQKAYQEIKQALLTAPALGLPDLTKPFELFVDEKQGYAKGVLTQKLGPWRRPVAYLSKKLDPVAAGWPPCLRMVAAIAVLTKDAGKLTMGQPLVILAPHAVEALVKQPPDRWLSNARMTHYQALLLDTDRVQFGPIVALNPATLLPLPEEGLQHDCLDILAEAHGTRPDLTDQPLPDADHTWYTDGSSFLQEGQRKAGAAVTTETEVVWAKALPAGTSAQRAELIALTQALKMAEGKKLNVYTDSRYAFATAHIHGEIYRRRGLLTSEGKEIKNKDEILALLKALFLPKRLSIIHCPGHQKGNRAEARGNRMADQAAREVATRETPETSTLLIENSAPYTHEHFHYTVTDIKDLTKLGATYDDAKKCWVYQGKPVMPDQFTFELLDFLHQLTHLSFSKTKALLERNYCPYYMLNRDRTLKDITETCQACAQVNASKSAVKQGTRVRGHRPGTHWEIDFTEVKPGLYGYKYLLVFIDTFSGWVEAFPTKKETAKVVTKKLLEEIFPRFGMPQVLGTDNGPAFVSKVSQTVADLLGVDWKLHCAYRPQSSGQVERMNRTIKETLTKLTLATGSRDWVLLLPLALYRARNTPGPHGLTPYEILYGAPPPLVNFPDPDMAKVTHNPSLQAHLQALYLVQHEVWRPLAAAYQEQLDRPVVPHPFRVGDTVWVRRHQTKNLEPRWKGPYTVLLTTPTALKVDGIAAWIHAAHVKAADTRIEPPSESTWRVQRSQNPLKIRLTRGTS

SEQ ID NO: 25 - protein, 546 aa, Baboon endogenous retrovirus
  BAEV-G protein
  BAEV-G protein
MGFTTKIIFLYNLVLVYAGFDDPRKAIELVQKRYGRPCDCSGGQVSEPPSDRVSQVTCSGKTAYLMPDQRWKCKSIPKDTSPSGPLQECPCNSYQSSVHSSCYTSYQQCRSGNKTYYTATLLKTQTGGTSDVQVLGSTNKLIQSPCNGIKGQSICWSTTAPIHVSDGGGPLDTTRIKSVQRKLEEIHKALYPELQYHPLAIPKVRDNLMVDAQTLNILNATYNLLLMSNTSLVDDCWLCLKLGPPTPLAIPNFLLSYVTRSSDNISCLIIPPLLVQPMQFSNSSCLFSPSYNSTEEIDLGHVAFSNCTSITNVTGPICAVNGSVFLCGNNMAYTYLPTNWTGLCVLATLLPDIDIIPGDEPVPIPAIDHFIYRPKRAIQFIPLLAGLGITAAFTTGATGLGVSVTQYTKLSNQLISDVQILSSTIQDLQDQVDSLAEVVLQNRRGLDLLTAEQGGICLALQEKCCFYVNKSGIVRDKIKTLQEELERRRKDLASNPLWTGLQGLLPYLLPFLGPLLTLLLLLTIGPCIFNRLTAFINDKLNIIHAM

SEQ ID NO: 26 - DNA, 5877 bp, Artificial Sequence
  sequence encoding Gag-Cas9 fusion protein
  sequence encoding Gag-Cas9 fusion protein
atgggccaggctgttaccacccccttaagtttgactttagaccactggaaggatgtcgaacggacagcccacaacctgtcggtagaggttagaaaaaggcgctgggttacattctgctctgcagaatggccaaccttcaacgtcggatggccacgagacggcacttttaacccagacattattacacaggttaagatcaaggtcttctcacctggcccacatggacatccggatcaggtcccctacatcgtgacctgggaagctatagcagtagacccccctccctgggtcagacccttcgtgcaccctaaacctcccctctctcttcccccttcagccccctctctcccacctgaacccccactctcgaccccgccccagtcctccctctatccggctctcacttctcctttaaacaccaaacctaggcctcaagtccttcctgatagcggaggaccactcattgatctactcacggaggaccctccgccttaccgggacccagggccaccctctcctgacgggaacggcgatagcggagaagtggcccctacagaaggagcccctgacccttccccaatggtatcccgcctgcggggaagaaaagaaccccccgtggcggattctactacctctcaggcgttcccccttcgcctgggagggaatggacagtatcaatactggccattttcctcctctgacctctataactggaaaaataacaacccctctttctccgaggacccagctaaattgacagctttgatcgagtccgttctccttactcatcagcccacttgggatgactgccaacagctattagggaccctgctgacgggagaagaaaaacagcgagtgctcctagaggcccgaaaggcggttcgaggggaggacggacgcccaactcagctgcccaatgacattaatgatgcttttcccttggaacgtcccgactgggactacaacacccaacgaggtaggaaccacctagtccactatcgccagttgctcctagcgggtctccaaaacgcgggcagaagccccaccaatttggccaaggtaaaagggataacccagggacctaatgagtctccctcagcctttttagagagactcaaggaggcctatcgcagatacactccttatgaccctgaggacccagggcaagaaaccaatgtggccatgtcattcatctggcagtccgccccggatatcgggcgaaagttagagcggttagaagatttgaagagtaagaccttaggagacttagtgagggaagctgaaaagatctttaataaacgagaaaccccggaagaaagagaggaacgtattaggagagaaacagaggaaaaggaagaacgccgtagggcagaggatgtgcagagagagaaggagagggaccgcagaagacatagagaaatgagtaagttgctggctactgtcgttagcgggcagagacaggatagacagggaggagagcgaaggaggccccaactcgaccacgaccagtgtgcctactgcaaagaaaagggacattgggctagagattgccccaagaagccaagaggaccccggggaccacgaccccaggcctccctcctgacgcgtagttccctgtatccagccctcacacctaccggtgattacaaagacgatgacgataagatggccccaaagaagaagcggaaggtcggtatccacggagtcccagcagccgacaagaagtacagcatcggcctggacatcggcaccaactctgtgggctgggccgtgatcaccgacgagtacaaggtgcccagcaagaaattcaaggtgctgggcaacaccgaccggcacagcatcaagaagaacctgatcggagccctgctgttcgacagcggcgaaacagccgaggccacccggctgaagagaaccgccagaagaagatacaccagacggaagaaccggatctgctatctgcaagagatcttcagcaacgagatggccaaggtggacgacagcttcttccacagactggaagagtccttcctggtggaagaggataagaagcacgagcggcaccccatcttcggcaacatcgtggacgaggtggcctaccacgagaagtaccccaccatctaccacctgagaaagaaactggtggacagcaccgacaaggccgacctgcggctgatctatctggccctggcccacatgatcaagttccggggccacttcctgatcgagggcgacctgaaccccgacaacagcgacgtggacaagctgttcatccagctggtgcagacctacaaccagctgttcgaggaaaaccccatcaacgccagcggcgtggacgccaaggccatcctgtctgccagactgagcaagagcagacggctggaaaatctgatcgcccagctgcccggcgagaagaagaatggcctgttcggcaacctgattgccctgagcctgggcctgacccccaacttcaagagcaacttcgacctggccgaggatgccaaactgcagctgagcaaggacacctacgacgacgacctggacaacctgctggcccagatcggcgaccagtacgccgacctgtttctggccgccaagaacctgtccgacgccatcctgctgagcgacatcctgagagtgaacaccgagatcaccaaggcccccctgagcgcctctatgatcaagagatacgacgagcaccaccaggacctgaccctgctgaaagctctcgtgcggcagcagctgcctgagaagtacaaagagattttcttcgaccagagcaagaacggctacgccggctacattgacggcggagccagccaggaagagttctacaagttcatcaagcccatcctggaaaagatggacggcaccgaggaactgctcgtgaagctgaacagagaggacctgctgcggaagcagcggaccttcgacaacggcagcatcccccaccagatccacctgggagagctgcacgccattctgcggcggcaggaagatttttacccattcctgaaggacaaccgggaaaagatcgagaagatcctgaccttccgcatcccctactacgtgggccctctggccaggggaaacagcagattcgcctggatgaccagaaagagcgaggaaaccatcaccccctggaacttcgaggaagtggtggacaagggcgcttccgcccagagcttcatcgagcggatgaccaacttcgataagaacctgcccaacgagaaggtgctgcccaagcacagcctgctgtacgagtacttcaccgtgtataacgagctgaccaaagtgaaatacgtgaccgagggaatgagaaagcccgccttcctgagcggcgagcagaaaaaggccatcgtggacctgctgttcaagaccaaccggaaagtgaccgtgaagcagctgaaagaggactacttcaagaaaatcgagtgcttcgactccgtggaaatctccggcgtggaagatcggttcaacgcctccctgggcacataccacgatctgctgaaaattatcaaggacaaggacttcctggacaatgaggaaaacgaggacattctggaagatatcgtgctgaccctgacactgtttgaggacagagagatgatcgaggaacggctgaaaacctatgcccacctgttcgacgacaaagtgatgaagcagctgaagcggcggagatacaccggctggggcaggctgagccggaagctgatcaacggcatccgggacaagcagtccggcaagacaatcctggatttcctgaagtccgacggcttcgccaacagaaacttcatgcagctgatccacgacgacagcctgacctttaaagaggacatccagaaagcccaggtgtccggccagggcgatagcctgcacgagcacattgccaatctggccggcagccccgccattaagaagggcatcctgcagacagtgaaggtggtggacgagctcgtgaaagtgatgggccggcacaagcccgagaacatcgtgatcgaaatggccagagagaaccagaccacccagaagggacagaagaacagccgcgagagaatgaagcggatcgaagagggcatcaaagagctgggcagccagatcctgaaagaacaccccgtggaaaacacccagctgcagaacgagaagctgtacctgtactacctgcagaatgggcgggatatgtacgtggaccaggaactggacatcaaccggctgtccgactacgatgtggaccatatcgtgcctcagagctttctgaaggacgactccatcgacaacaaggtgctgaccagaagcgacaagaaccggggcaagagcgacaacgtgccctccgaagaggtcgtgaagaagatgaagaactactggcggcagctgctgaacgccaagctgattacccagagaaagttcgacaatctgaccaaggccgagagaggcggcctgagcgaactggataaggccggcttcatcaagagacagctggtggaaacccggcagatcacaaagcacgtggcacagatcctggactcccggatgaacactaagtacgacgagaatgacaagctgatccgggaagtgaaagtgatcaccctgaagtccaagctggtgtccgatttccggaaggatttccagttttacaaagtgcgcgagatcaacaactaccaccacgcccacgacgcctacctgaacgccgtcgtgggaaccgccctgatcaaaaagtaccctaagctggaaagcgagttcgtgtacggcgactacaaggtgtacgacgtgcggaagatgatcgccaagagcgagcaggaaatcggcaaggctaccgccaagtacttcttctacagcaacatcatgaactttttcaagaccgagattaccctggccaacggcgagatccggaagcggcctctgatcgagacaaacggcgaaaccggggagatcgtgtgggataagggccgggattttgccaccgtgcggaaagtgctgagcatgccccaagtgaatatcgtgaaaaagaccgaggtgcagacaggcggcttcagcaaagagtctatcctgcccaagaggaacagcgataagctgatcgccagaaagaaggactgggaccctaagaagtacggcggcttcgacagccccaccgtggcctattctgtgctggtggtggccaaagtggaaaagggcaagtccaagaaactgaagagtgtgaaagagctgctggggatcaccatcatggaaagaagcagcttcgagaagaatcccatcgactttctggaagccaagggctacaaagaagtgaaaaaggacctgatcatcaagctgcctaagtactccctgttcgagctggaaaacggccggaagagaatgctggcctctgccggcgaactgcagaagggaaacgaactggccctgccctccaaatatgtgaacttcctgtacctggccagccactatgagaagctgaagggctcccccgaggataatgagcagaaacagctgtttgtggaacagcacaagcactacctggacgagatcatcgagcagatcagcgagttctccaagagagtgatcctggccgacgctaatctggacaaagtgctgtccgcctacaacaagcaccgggataagcccatcagagagcaggccgagaatatcatccacctgtttaccctgaccaatctgggagcccctgccgccttcaagtactttgacaccaccatcgaccggaagaggtacaccagcaccaaagaggtgctggacgccaccctgatccaccagagcatcaccggcctgtacgagacacggatcgacctgtctcagctgggaggcgacaagcgtcctgctgctactaagaaagctggtcaagctaagaaaaagaaagctagagcttga

SEQ ID NO: 27 - DNA, 1641 bp, baboon endogenous retrovirus
  sequence encoding BAEV-G
  sequence encoding BAEV-G
atgggctttaccaccaagattatttttctgtataacctggtgctggtgtatgcgggctttgatgatccgcgcaaagcgattgaactggtgcagaaacgctatggccgcccgtgcgattgcagcggcggccaggtgagcgaaccgccgagcgatcgcgtgagccaggtgacctgcagcggcaaaaccgcgtatctgatgccggatcagcgctggaaatgcaaaagcattccgaaagataccagcccgagcggcccgctgcaggaatgcccgtgcaacagctatcagagcagcgtgcatagcagctgctataccagctatcagcagtgccgcagcggcaacaaaacctattataccgcgaccctgctgaaaacccagaccggcggcaccagcgatgtgcaggtgctgggcagcaccaacaaactgattcagagcccgtgcaacggcattaaaggccagagcatttgctggagcaccaccgcgccgattcatgtgagcgatggcggcggcccgctggataccacccgcattaaaagcgtgcagcgcaaactggaagaaattcataaagcgctgtatccggaactgcagtatcatccgctggcgattccgaaagtgcgcgataacctgatggtggatgcgcagaccctgaacattctgaacgcgacctataacctgctgctgatgagcaacaccagcctggtggatgattgctggctgtgcctgaaactgggcccgccgaccccgctggcgattccgaactttctgctgagctatgtgacccgcagcagcgataacattagctgcctgattattccgccgctgctggtgcagccgatgcagtttagcaacagcagctgcctgtttagcccgagctataacagcaccgaagaaattgatctgggccatgtggcgtttagcaactgcaccagcattaccaacgtgaccggcccgatttgcgcggtgaacggcagcgtgtttctgtgcggcaacaacatggcgtatacctatctgccgaccaactggaccggcctgtgcgtgctggcgaccctgctgccggatattgatattattccgggcgatgaaccggtgccgattccggcgattgatcattttatttatcgcccgaaacgcgcgattcagtttattccgctgctggcgggcctgggcattaccgcggcgtttaccaccggcgcgaccggcctgggcgtgagcgtgacccagtataccaaactgagcaaccagctgattagcgatgtgcagattctgagcagcaccattcaggatctgcaggatcaggtggatagcctggcggaagtggtgctgcagaaccgccgcggcctggatctgctgaccgcggaacagggcggcatttgcctggcgctgcaggaaaaatgctgcttttatgtgaacaaaagcggcattgtgcgcgataaaattaaaaccctgcaggaagaactggaacgccgccgcaaagatctggcgagcaacccgctgtggaccggcctgcagggcctgctgccgtatctgctgccgtttctgggcccgctgctgaccctgctgctgctgctgaccattggcccgtgcatttttaaccgcctgaccgcgtttattaacgataaactgaacattattcatgcgatgtaa

SEQ ID NO: 28 - DNA, 1536 bp, Vesicular stomatitis virus
  sequence encoding VSV-G protein
  sequence encoding VSV-G protein
atgaagtgccttttgtacttagcctttttattcattggggtgaattgcaagttcaccatagtttttccacacaaccaaaaaggaaactggaaaaatgttccttctaattaccattattgcccgtcaagctcagatttaaattggcataatgacttaataggcacagccttacaagtcaaaatgcccaagagtcacaaggctattcaagcagacggttggatgtgtcatgcttccaaatgggtcactacttgtgatttccgctggtatggaccgaagtatataacacattccatccgatccttcactccatctgtagaacaatgcaaggaaagcattgaacaaacgaaacaaggaacttggctgaatccaggcttccctcctcaaagttgtggatatgcaactgtgacggatgccgaagcagtgattgtccaggtgactcctcaccatgtgctggttgatgaatacacaggagaatgggttgattcacagttcatcaacggaaaatgcagcaattacatatgccccactgtccataactctacaacctggcattctgactataaggtcaaagggctatgtgattctaacctcatttccatggacatcaccttcttctcagaggacggagagctatcatccctgggaaaggagggcacagggttcagaagtaactactttgcttatgaaactggaggcaaggcctgcaaaatgcaatactgcaagcattggggagtcagactcccatcaggtgtctggttcgagatggctgataaggatctctttgctgcagccagattccctgaatgcccagaagggtcaagtatctctgctccatctcagacctcagtggatgtaagtctaattcaggacgttgagaggatcttggattattccctctgccaagaaacctggagcaaaatcagagcgggtcttccaatctctccagtggatctcagctatcttgctcctaaaaacccaggaaccggtcctgctttcaccataatcaatggtaccctaaaatactttgagaccagatacatcagagtcgatattgctgctccaatcctctcaagaatggtcggaatgatcagtggaactaccacagaaagggaactgtgggatgactgggcaccatatgaagacgtggaaattggacccaatggagttctgaggaccagttcaggatataagtttcctttatacatgattggacatggtatgttggactccgatcttcatcttagctcaaaggctcaggtgttcgaacatcctcacattcaagacgctgcttcgcaacttcctgatgatgagagtttattttttggtgatactgggctatccaaaaatccaatcgagcttgtagaaggttggttcagtagttggaaaagctctattgcctcttttttctttatcatagggttaatcattggactattcttggttctccgagttggtatccatctttgcattaaattaaagcacaccaagaaaagacagatttatacagacatagagatgaaccgacttggaaagtaa

SEQ ID NO: 29 - protein, 9 aa, Artificial Sequence
  cleavage sequence
  cleavage sequence
SSLYPALTP

SEQ ID NO: 30 - DNA, 27 bp, Artificial Sequence
  sequence encoding the cleavage sequence of SEQ ID NO. 29
  sequence encoding the cleavage sequence of SEQ ID NO. 29
agttccctgtatccagccctcacacct

SEQ ID NO: 31 - protein, 1401 aa, Streptococcus
  Cas9
  Cas9
MAPKKKRKVGIHGVPAADKKYSIGLDIGTNSVGWAVITDEYKVPSKKFKVLGNTDRHSIKKNLIGALLFDSGETAEATRLKRTARRRYTRRKNRICYLQEIFSNEMAKVDDSFFHRLEESFLVEEDKKHERHPIFGNIVDEVAYHEKYPTIYHLRKKLVDSTDKADLRLIYLALAHMIKFRGHFLIEGDLNPDNSDVDKLFIQLVQTYNQLFEENPINASGVDAKAILSARLSKSRRLENLIAQLPGEKKNGLFGNLIALSLGLTPNFKSNFDLAEDAKLQLSKDTYDDDLDNLLAQIGDQYADLFLAAKNLSDAILLSDILRVNTEITKAPLSASMIKRYDEHHQDLTLLKALVRQQLPEKYKEIFFDQSKNGYAGYIDGGASQEEFYKFIKPILEKMDGTEELLVKLNREDLLRKQRTFDNGSIPHQIHLGELHAILRRQEDFYPFLKDNREKIEKILTFRIPYYVGPLARGNSRFAWMTRKSEETITPWNFEEVVDKGASAQSFIERMTNFDKNLPNEKVLPKHSLLYEYFTVYNELTKVKYVTEGMRKPAFLSGEQKKAIVDLLFKTNRKVTVKQLKEDYFKKIECFDSVEISGVEDRFNASLGTYHDLLKIIKDKDFLDNEENEDILEDIVLTLTLFEDREMIEERLKTYAHLFDDKVMKQLKRRRYTGWGRLSRKLINGIRDKQSGKTILDFLKSDGFANRNFMQLIHDDSLTFKEDIQKAQVSGQGDSLHEHIANLAGSPAIKKGILQTVKVVDELVKVMGRHKPENIVIEMARENQTTQKGQKNSRERMKRIEEGIKELGSQILKEHPVENTQLQNEKLYLYYLQNGRDMYVDQELDINRLSDYDVDHIVPQSFLKDDSIDNKVLTRSDKNRGKSDNVPSEEVVKKMKNYWRQLLNAKLITQRKFDNLTKAERGGLSELDKAGFIKRQLVETRQITKHVAQILDSRMNTKYDENDKLIREVKVITLKSKLVSDFRKDFQFYKVREINNYHHAHDAYLNAVVGTALIKKYPKLESEFVYGDYKVYDVRKMIAKSEQEIGKATAKYFFYSNIMNFFKTEITLANGEIRKRPLIETNGETGEIVWDKGRDFATVRKVLSMPQVNIVKKTEVQTGGFSKESILPKRNSDKLIARKKDWDPKKYGGFDSPTVAYSVLVVAKVEKGKSKKLKSVKELLGITIMERSSFEKNPIDFLEAKGYKEVKKDLIIKLPKYSLFELENGRKRMLASAGELQKGNELALPSKYVNFLYLASHYEKLKGSPEDNEQKQLFVEQHKHYLDEIIEQISEFSKRVILADANLDKVLSAYNKHRDKPIREQAENIIHLFTLTNLGAPAAFKYFDTTIDRKRYTSTKEVLDATLIHQSITGLYETRIDLSQLGGDKRPAATKKAGQAKKKKA

SEQ ID NO: 32 - DNA, 4205 bp, Streptococcus
  encoding Cas9
  encoding Cas9
atggccccaaagaagaagcggaaggtcggtatccacggagtcccagcagccgacaagaagtacagcatcggcctggacatcggcaccaactctgtgggctgggccgtgatcaccgacgagtacaaggtgcccagcaagaaattcaaggtgctgggcaacaccgaccggcacagcatcaagaagaacctgatcggagccctgctgttcgacagcggcgaaacagccgaggccacccggctgaagagaaccgccagaagaagatacaccagacggaagaaccggatctgctatctgcaagagatcttcagcaacgagatggccaaggtggacgacagcttcttccacagactggaagagtccttcctggtggaagaggataagaagcacgagcggcaccccatcttcggcaacatcgtggacgaggtggcctaccacgagaagtaccccaccatctaccacctgagaaagaaactggtggacagcaccgacaaggccgacctgcggctgatctatctggccctggcccacatgatcaagttccggggccacttcctgatcgagggcgacctgaaccccgacaacagcgacgtggacaagctgttcatccagctggtgcagacctacaaccagctgttcgaggaaaaccccatcaacgccagcggcgtggacgccaaggccatcctgtctgccagactgagcaagagcagacggctggaaaatctgatcgcccagctgcccggcgagaagaagaatggcctgttcggcaacctgattgccctgagcctgggcctgacccccaacttcaagagcaacttcgacctggccgaggatgccaaactgcagctgagcaaggacacctacgacgacgacctggacaacctgctggcccagatcggcgaccagtacgccgacctgtttctggccgccaagaacctgtccgacgccatcctgctgagcgacatcctgagagtgaacaccgagatcaccaaggcccccctgagcgcctctatgatcaagagatacgacgagcaccaccaggacctgaccctgctgaaagctctcgtgcggcagcagctgcctgagaagtacaaagagattttcttcgaccagagcaagaacggctacgccggctacattgacggcggagccagccaggaagagttctacaagttcatcaagcccatcctggaaaagatggacggcaccgaggaactgctcgtgaagctgaacagagaggacctgctgcggaagcagcggaccttcgacaacggcagcatcccccaccagatccacctgggagagctgcacgccattctgcggcggcaggaagatttttacccattcctgaaggacaaccgggaaaagatcgagaagatcctgaccttccgcatcccctactacgtgggccctctggccaggggaaacagcagattcgcctggatgaccagaaagagcgaggaaaccatcaccccctggaacttcgaggaagtggtggacaagggcgcttccgcccagagcttcatcgagcggatgaccaacttcgataagaacctgcccaacgagaaggtgctgcccaagcacagcctgctgtacgagtacttcaccgtgtataacgagctgaccaaagtgaaatacgtgaccgagggaatgagaaagcccgccttcctgagcggcgagcagaaaaaggccatcgtggacctgctgttcaagaccaaccggaaagtgaccgtgaagcagctgaaagaggactacttcaagaaaatcgagtgcttcgactccgtggaaatctccggcgtggaagatcggttcaacgcctccctgggcacataccacgatctgctgaaaattatcaaggacaaggacttcctggacaatgaggaaaacgaggacattctggaagatatcgtgctgaccctgacactgtttgaggacagagagatgatcgaggaacggctgaaaacctatgcccacctgttcgacgacaaagtgatgaagcagctgaagcggcggagatacaccggctggggcaggctgagccggaagctgatcaacggcatccgggacaagcagtccggcaagacaatcctggatttcctgaagtccgacggcttcgccaacagaaacttcatgcagctgatccacgacgacagcctgacctttaaagaggacatccagaaagcccaggtgtccggccagggcgatagcctgcacgagcacattgccaatctggccggcagccccgccattaagaagggcatcctgcagacagtgaaggtggtggacgagctcgtgaaagtgatgggccggcacaagcccgagaacatcgtgatcgaaatggccagagagaaccagaccacccagaagggacagaagaacagccgcgagagaatgaagcggatcgaagagggcatcaaagagctgggcagccagatcctgaaagaacaccccgtggaaaacacccagctgcagaacgagaagctgtacctgtactacctgcagaatgggcgggatatgtacgtggaccaggaactggacatcaaccggctgtccgactacgatgtggaccatatcgtgcctcagagctttctgaaggacgactccatcgacaacaaggtgctgaccagaagcgacaagaaccggggcaagagcgacaacgtgccctccgaagaggtcgtgaagaagatgaagaactactggcggcagctgctgaacgccaagctgattacccagagaaagttcgacaatctgaccaaggccgagagaggcggcctgagcgaactggataaggccggcttcatcaagagacagctggtggaaacccggcagatcacaaagcacgtggcacagatcctggactcccggatgaacactaagtacgacgagaatgacaagctgatccgggaagtgaaagtgatcaccctgaagtccaagctggtgtccgatttccggaaggatttccagttttacaaagtgcgcgagatcaacaactaccaccacgcccacgacgcctacctgaacgccgtcgtgggaaccgccctgatcaaaaagtaccctaagctggaaagcgagttcgtgtacggcgactacaaggtgtacgacgtgcggaagatgatcgccaagagcgagcaggaaatcggcaaggctaccgccaagtacttcttctacagcaacatcatgaactttttcaagaccgagattaccctggccaacggcgagatccggaagcggcctctgatcgagacaaacggcgaaaccggggagatcgtgtgggataagggccgggattttgccaccgtgcggaaagtgctgagcatgccccaagtgaatatcgtgaaaaagaccgaggtgcagacaggcggcttcagcaaagagtctatcctgcccaagaggaacagcgataagctgatcgccagaaagaaggactgggaccctaagaagtacggcggcttcgacagccccaccgtggcctattctgtgctggtggtggccaaagtggaaaagggcaagtccaagaaactgaagagtgtgaaagagctgctggggatcaccatcatggaaagaagcagcttcgagaagaatcccatcgactttctggaagccaagggctacaaagaagtgaaaaaggacctgatcatcaagctgcctaagtactccctgttcgagctggaaaacggccggaagagaatgctggcctctgccggcgaactgcagaagggaaacgaactggccctgccctccaaatatgtgaacttcctgtacctggccagccactatgagaagctgaagggctcccccgaggataatgagcagaaacagctgtttgtggaacagcacaagcactacctggacgagatcatcgagcagatcagcgagttctccaagagagtgatcctggccgacgctaatctggacaaagtgctgtccgcctacaacaagcaccgggataagcccatcagagagcaggccgagaatatcatccacctgtttaccctgaccaatctgggagcccctgccgccttcaagtactttgacaccaccatcgaccggaagaggtacaccagcaccaaagaggtgctggacgccaccctgatccaccagagcatcaccggcctgtacgagacacggatcgacctgtctcagctgggaggcgacaagcgtcctgctgctactaagaaagctggtcaagctaagaaaaagaaagctag

SEQ ID NO: 33 - DNA, 12150 bp, Artificial Sequence
  HIV-1 encapsidation construct
  HIV-1 encapsidation construct
ttgattattgactagttattaatagtaatcaattacggggtcattagttcatagcccatatatggagttccgcgttacataacttacggtaaatggcccgcctggctgaccgcccaacgacccccgcccattgacgtcaataatgacgtatgttcccatagtaacgccaatagggactttccattgacgtcaatgggtggagtatttacggtaaactgcccacttggcagtacatcaagtgtatcatatgccaagtacgccccctattgacgtcaatgacggtaaatggcccgcctggcattatgcccagtacatgaccttatgggactttcctacttggcagtacatctacgtattagtcatcgctattaccatggtgatgcggttttggcagtacatcaatgggcgtggatagcggtttgactcacggggatttccaagtctccaccccattgacgtcaatgggagtttgttttggcaccaaaatcaacgggactttccaaaatgtcgtaacaactccgccccattgacgcaaatgggcggtaggcgtgtacggtgggaggtctatataagcagagctcgtttagtgaaccgtcagatcgcctggagacgccatccacgctgttttgacctccatagaagacaccgggaccgatccagcctccgcggccgggaacggtgcattggaacgcggattccccgtgccaagagtgacgtaagtaccgcctatagagtctataggcccacccccttggcttcttatgcgacggatcgatcccgtaataagcttcgaggtccgcggccggccgcgttgacgcgcacggcaagaggcgaggggcggcgactggtgagagatgggtgcgagagcgtcagtattaagcgggggagaattagatcgatgggaaaaaattcggttaaggccagggggaaagaaaaaatataaattaaaacatatagtatgggcaagcagggagctagaacgattcgcagttaatcctggcctgttagaaacatcagaaggctgtagacaaatactgggacagctacaaccatcccttcagacaggatcagaagaacttagatcattatataatacagtagcaaccctctattgtgtgcatcaaaggatagagataaaagacaccaaggaagctttagacaagatagaggaagagcaaaacaaaagtaagaaaaaagcacagcaagcagcagctgacacaggacacagcaatcaggtcagccaaaattaccctatagtgcagaacatccaggggcaaatggtacatcaggccatatcacctagaactttaaatgcatgggtaaaagtagtagaagagaaggctttcagcccagaagtgatacccatgttttcagcattatcagaaggagccaccccacaagatttaaacaccatgctaaacacagtggggggacatcaagcagccatgcaaatgttaaaagagaccatcaatgaggaagctgcagaatgggatagagtgcatccagtgcatgcagggcctattgcaccaggccagatgagagaaccaaggggaagtgacatagcaggaactactagtacccttcaggaacaaataggatggatgacacataatccacctatcccagtaggagaaatctataaaagatggataatcctgggattaaataaaatagtaagaatgtatagccctaccagcattctggacataagacaaggaccaaaggaaccctttagagactatgtagaccgattctataaaactctaagagccgagcaagcttcacaagaggtaaaaaattggatgacagaaaccttgttggtccaaaatgcgaacccagattgtaagactattttaaaagcattgggaccaggagcgacactagaagaaatgatgacagcatgtcagggagtggggggacccggccataaagcaagagttttggctgaagcaatgagccaagtaacaaatccagctaccataatgatacagaaaggcaattttaggaaccaaagaaagactgttaagtgtttcaattgtggcaaagaagggcacatagccaaaaattgcagggcccctaggaaaaagggctgttggaaatgtggaaaggaaggacaccaaatgaaagattgtactgagagacaggctaattttttagggaagatctggccttcccacaagggaaggccagggaattttcttcagagcagaccagagccaacagccccaccagaagagagcttcaggtttggggaagagacaacaactccctctcagaagcaggagccgatagacaaggaactgtatcctttagcttccctcagatcactctttggcagcgacccctcgtcacaataaagataggggggcaattaaaggaagctctattagatacaggagcagatgatacagtattagaagaaatgaatttgccaggaagatggaaaccaaaaatgatagggggaattggaggttttatcaaagtaagacagtatgatcagatactcatagaaatctgcggacataaagctataggtacagtattagtaggacctacacctgtcaacataattggaagaaatctgttgactcagattggctgcactttaaattttcccattagtcctattgagactgtaccagtaaaattaaagccaggaatggatggcccaaaagttaaacaatggccattgacagaagaaaaaataaaagcattagtagaaatttgtacagaaatggaaaaggaaggaaaaatttcaaaaattgggcctgaaaatccatacaatactccagtatttgccataaagaaaaaagacagtactaaatggagaaaattagtagatttcagagaacttaataagagaactcaagatttctgggaagttcaattaggaataccacatcctgcagggttaaaacagaaaaaatcagtaacagtactggatgtgggcgatgcatatttttcagttcccttagataaagacttcaggaagtatactgcatttaccatacctagtataaacaatgagacaccagggattagatatcagtacaatgtgcttccacagggatggaaaggatcaccagcaatattccagtgtagcatgacaaaaatcttagagccttttagaaaacaaaatccagacatagtcatctatcaatacatggatgatttgtatgtaggatctgacttagaaatagggcagcatagaacaaaaatagaggaactgagacaacatctgttgaggtggggatttaccacaccagacaaaaaacatcagaaagaacctccattcctttggatgggttatgaactccatcctgataaatggacagtacagcctatagtgctgccagaaaaggacagctggactgtcaatgacatacagaaattagtgggaaaattgaattgggcaagtcagatttatgcagggattaaagtaaggcaattatgtaaacttcttaggggaaccaaagcactaacagaagtagtaccactaacagaagaagcagagctagaactggcagaaaacagggagattctaaaagaaccggtacatggagtgtattatgacccatcaaaagacttaatagcagaaatacagaagcaggggcaaggccaatggacatatcaaatttatcaagagccatttaaaaatctgaaaacaggaaagtatgcaagaatgaagggtgcccacactaatgatgtgaaacaattaacagaggcagtacaaaaaatagccacagaaagcatagtaatatggggaaagactcctaaatttaaattacccatacaaaaggaaacatgggaagcatggtggacagagtattggcaagccacctggattcctgagtgggagtttgtcaatacccctcccttagtgaagttatggtaccagttagagaaagaacccataataggagcagaaactttctatgtagatggggcagccaatagggaaactaaattaggaaaagcaggatatgtaactgacagaggaagacaaaaagttgtccccctaacggacacaacaaatcagaagactgagttacaagcaattcatctagctttgcaggattcgggattagaagtaaacatagtgacagactcacaatatgcattgggaatcattcaagcacaaccagataagagtgaatcagagttagtcagtcaaataatagagcagttaataaaaaaggaaaaagtctacctggcatgggtaccagcacacaaaggaattggaggaaatgaacaagtagataaattggtcagtgctggaatcaggaaagtactatttttagatggaatagataaggcccaagaagaacatgagaaatatcacagtaattggagagcaatggctagtgattttaacctaccacctgtagtagcaaaagaaatagtagccagctgtgataaatgtcagctaaaaggggaagccatgcatggacaagtagactgtagcccaggaatatggcagctagattgtacacatttagaaggaaaagttatcttggtagcagttcatgtagccagtggatatatagaagcagaagtaattccagcagagacagggcaagaaacagcatacttcctcttaaaattagcaggaagatggccagtaaaaacagtacatacagacaatggcagcaatttcaccagtactacagttaaggccgcctgttggtgggcggggatcaagcaggaatttggcattccctacaatccccaaagtcaaggagtaatagaatctatgaataaagaattaaagaaaattataggacaggtaagagatcaggctgaacatcttaagacagcagtacaaatggcagtattcatccacaattttaaaagaaaaggggggattggggggtacagtgcaggggaaagaatagtagacataatagcaacagacatacaaactaaagaattacaaaaacaaattacaaaaattcaaaattttcgggtttattacagggacagcagagatccagtttggaaaggaccagcaaagctcctctggaaaggtgaaggggcagtagtaatacaagataatagtgacataaaagtagtgccaagaagaaaagcaaagatcatcagggattatggaaaacagatggcaggtgatgattgtgtggcaagtagacaggatgaggattaacacatggaattctgcaacaactgctgtttatccatttcagaattgggtgtcgacatagcagaataggcgttactcgacagaggagagcaagaaatggagccagtagatcctagactagagccctggaagcatccaggaagtcagcctaaaactgcttgtaccaattgctattgtaaaaagtgttgctttcattgccaagtttgtttcatgacaaaagccttaggcatctcctatggcaggaagaagcggagacagcgacgaagagctcatcagaacagtcagactcatcaagcttctctatcaaagcagtaagtagtacatgtaatgcaacctataatagtagcaatagtagcattagtagtagcaataataatagcaatagttgtgtggtccatagtaatcatagaatataggaaaatggccgctgatcttcagacctggaggaggagatatgagggacaattggagaagtgaattatataaatataaagtagtaaaaattgaaccattaggagtagcacccaccaaggcaaagagaagagtggtgcagagagaaaaaagagcagtgggaataggagctttgttccttgggttcttgggagcagcaggaagcactatgggcgcagcgtcaatgacgctgacggtacaggccagacaattattgtctggtatagtgcagcagcagaacaatttgctgagggctattgaggcgcaacagcatctgttgcaactcacagtctggggcatcaagcagctccaggcaagaatcctggctgtggaaagatacctaaaggatcaacagctcctggggatttggggttgctctggaaaactcatttgcaccactgctgtgccttggaatgctagttggagtaataaatctctggaacagatttggaatcacacgacctggatggagtgggacagagaaattaacaattacacaagcttaatacactccttaattgaagaatcgcaaaaccagcaagaaaagaatgaacaagaattattggaattagataaatgggcaagtttgtggaattggtttaacataacaaattggctgtggtatataaaattattcataatgatagtaggaggcttggtaggtttaagaatagtttttgctgtactttctatagtgaatagagttaggcagggatattcaccattatcgtttcagacccacctcccaaccccgaggggacccgacaggcccgaaggaatagaagaagaaggtggagagagagacagagacagatccattcgattagtgaacggatccttggcacttatctgggacgatctgcggagcctgtgcctcttcagctaccaccgcttgagagacttactcttgattgtaacgaggattgtggaacttctgggacgcagggggtgggaagccctcaaatattggtggaatctcctacaatattggagtcaggagctaaagaatagtgctgttagcttgctcaatgccacagccatagcagtagctgaggggacagatagggttatagaagtagtacaaggagcttgtagagctattcgccacatacctagaagaataagacagggcttggaaaggattttgctataagctcgaggccgccccggtgaccttcagaccttggcactggaggtggcccggcagaagcgcggcatcgtggatcagtgctgcaccagcatctgctctctctaccaactggagaactactgcaactaggcccaccactaccctgtccacccctctgcaatgaataaaacctttgaaagagcactacaagttgtgtgtacatgcgtgcatgtgcatatgtggtgcggggggaacatgagtggggctggctggagtggcgatgataagctgtcaaacatgagaattaattcttgaagacgaaagggcctcgtgatacgcctatttttataggttaatgtcatgataataatggtttcttagtctagaattaattccgtgtattctatagtgtcacctaaatcgtatgtgtatgatacataaggttatgtattaattgtagccgcgttctaacgacaatatgtacaagcctaattgtgtagcatctggcttactgaagcagaccctatcatctctctcgtaaactgccgtcagagtcggtttggttggacgaaccttctgagtttctggtaacgccgtcccgcacccggaaatggtcagcgaaccaatcagcagggtcatcgctagccagatcctctacgccggacgcatcgtggccggcatcaccggcgccacaggtgcggttgctggcgcctatatcgccgacatcaccgatggggaagatcgggctcgccacttcgggctcatgagcgcttgtttcggcgtgggtatggtggcaggccccgtggccgggggactgttgggcgccatctccttgcatgcaccattccttgcggcggcggtgctcaacggcctcaacctactactgggctgcttcctaatgcaggagtcgcataagggagagcgtcgaatggtgcactctcagtacaatctgctctgatgccgcatagttaagccagccccgacacccgccaacacccgctgacgcgccctgacgggcttgtctgctcccggcatccgcttacagacaagctgtgaccgtctccgggagctgcatgtgtcagaggttttcaccgtcatcaccgaaacgcgcgagacgaaagggcctcgtgatacgcctatttttataggttaatgtcatgataataatggtttcttagacgtcaggtggcacttttcggggaaatgtgcgcggaacccctatttgtttatttttctaaatacattcaaatatgtatccgctcatgagacaataaccctgataaatgcttcaataatattgaaaaaggaagagtatgagtattcaacatttccgtgtcgcccttattcccttttttgcggcattttgccttcctgtttttgctcacccagaaacgctggtgaaagtaaaagatgctgaagatcagttgggtgcacgagtgggttacatcgaactggatctcaacagcggtaagatccttgagagttttcgccccgaagaacgttttccaatgatgagcacttttaaagttctgctatgtggcgcggtattatcccgtattgacgccgggcaagagcaactcggtcgccgcatacactattctcagaatgacttggttgagtactcaccagtcacagaaaagcatcttacggatggcatgacagtaagagaattatgcagtgctgccataaccatgagtgataacactgcggccaacttacttctgacaacgatcggaggaccgaaggagctaaccgcttttttgcacaacatgggggatcatgtaactcgccttgatcgttgggaaccggagctgaatgaagccataccaaacgacgagcgtgacaccacgatgcctgtagcaatggcaacaacgttgcgcaaactattaactggcgaactacttactctagcttcccggcaacaattaatagactggatggaggcggataaagttgcaggaccacttctgcgctcggcccttccggctggctggtttattgctgataaatctggagccggtgagcgtgggtctcgcggtatcattgcagcactggggccagatggtaagccctcccgtatcgtagttatctacacgacggggagtcaggcaactatggatgaacgaaatagacagatcgctgagataggtgcctcactgattaagcattggtaactgtcagaccaagtttactcatatatactttagattgatttaaaacttcatttttaatttaaaaggatctaggtgaagatcctttttgataatctcatgaccaaaatcccttaacgtgagttttcgttccactgagcgtcagaccccgtagaaaagatcaaaggatcttcttgagatcctttttttctgcgcgtaatctgctgcttgcaaacaaaaaaaccaccgctaccagcggtggtttgtttgccggatcaagagctaccaactctttttccgaaggtaactggcttcagcagagcgcagataccaaatactgttcttctagtgtagccgtagttaggccaccacttcaagaactctgtagcaccgcctacatacctcgctctgctaatcctgttaccagtggctgctgccagtggcgataagtcgtgtcttaccgggttggactcaagacgatagttaccggataaggcgcagcggtcgggctgaacggggggttcgtgcacacagcccagcttggagcgaacgacctacaccgaactgagatacctacagcgtgagctatgagaaagcgccacgcttcccgaagggagaaaggcggacaggtatccggtaagcggcagggtcggaacaggagagcgcacgagggagcttccagggggaaacgcctggtatctttatagtcctgtcgggtttcgccacctctgacttgagcgtcgatttttgtgatgctcgtcaggggggcggagcctatggaaaaacgccagcaacgcggcctttttacggttcctggccttttgctggccttttgctcacatgttctttcctgcgttatcccctgattctgtggataaccgtattaccgcctttgagtgagctgataccgctcgccgcagccgaacgaccgagcgcagcgagtcagtgagcgaggaagcggaagagcgcccaatacgcaaaccgcctctccccgcgcgttggccgattcattaatgcagctgtggaatgtgtgtcagttagggtgtggaaagtccccaggctccccagcaggcagaagtatgcaaagcatgcatctcaattagtcagcaaccaggtgtggaaagtccccaggctccccagcaggcagaagtatgcaaagcatgcatctcaattagtcagcaaccatagtcccgcccctaactccgcccatcccgcccctaactccgcccagttccgcccattctccgccccatggctgactaattttttttatttatgcagaggccgaggccgcctcggcctctgagctattccagaagtagtgaggaggcttttttggaggcctaggcttttgcaaaaagcttggacacaagacaggcttgcgagatatgtttgagaataccactttatcccgcgtcagggagaggcagtgcgtaaaaagacgcggactcatgtgaaatactggtttttagtgcgccagatctctataatctcgcgcaacctattttcccctcgaacactttttaagccgtagataaacaggctgggacacttcacatgagcgaaaaatacatcgtcacctgggacatgttgcagatccatgcacgtaaactcgcaagccgactgatgccttctgaacaatggaaaggcattattgccgtaagccgtggcggtctgtaccgggtgcgttactggcgcgtgaactgggtattcgtcatgtcgataccgtttgtatttccagctacgatcacgacaaccagcgcgagcttaaagtgctgaaacgcgcagaaggcgatggcgaaggcttcatcgttattgatgacctggtggataccggtggtactgcggttgcgattcgtgaaatgtatccaaaagcgcactttgtcaccatcttcgcaaaaccggctggtcgtccgctggttgatgactatgttgttgatatcccgcaagatacctggattgaacagccgtgggatatgggcgtcgtattcgtcccgccaatctccggtcgctaatcttttcaacgcctggcactgccgggcgttgttctttttaacttcaggcgggttacaatagtttccagtaagtattctggaggctgcatccatgacacaggcaaacctgagcgaaaccctgttcaaaccccgctttaaacatcctgaaacctcgacgctagtccgccgctttaatcacggcgcacaaccgcctgtgcagtcggcccttgatggtaaaaccatccctcactggtatcgcatgattaaccgtctgatgtggatctggcgcggcattgacccacgcgaaatcctcgacgtccaggcacgtattgtgatgagcgatgccgaacgtaccgacgatgatttatacgatacggtgattggctaccgtggcggcaactggatttatgagtgggccccggatctttgtgaaggaaccttacttctgtggtgtgacataattggacaaactacctacagagatttaaagctctaaggtaaatataaaatttttaacccggatctttgtgaaggaaccttacttctgtggtgtgacataattggacaaactacctacagagatttaaagctctaaggtaaatataaaatttttaagtgtataatgtgttaaactactgattctaattgtttgtgtattttagattccaacctatggaactgatgaatgggagcagtggtggaatgcctttaatgaggaaaacctgttttgctcagaagaaatgccatctagtgatgatgaggctactgctgactctcaacattctactcctccaaaaaagaagagaaaggtagaagaccccaaggactttccttcagaattgctaagttttttgagtcatgctgtgtttagtaatagaactcttgcttgctttgctatttacaccacaaaggaaaaagctgcactgctatacaagaaaattatggaaaaatattctgtaacctttataagtaggcataacagttataatcataacatactgttttttcttactccacacaggcatagagtgtctgctattaataactatgctcaaaaattgtgtacctttagctttttaatttgtaaaggggttaataaggaatatttgatgtatagtgccttgactagagatcataatcagccataccacatttgtagaggttttacttgctttaaaaaacctcccacacctccccctgaacctgaaacataaaatgaatgcaattgttgttgttgggctgcaggaattaattcgagctcgcccgaca

SEQ ID NO: 34 - DNA, 10627 bp, Artificial Sequence
  encoding HIV-1 GAG-CAS9 construct
  encoding HIV-1 GAG-CAS9 construct
gcggccgctctagagagcttggcccattgcatacgttgtatccatatcataatatgtacatttatattggctcatgtccaacattaccgccatgttgacattgattattgactagttattaatagtaatcaattacggggtcattagttcatagcccatatatggagttccgcgttacataacttacggtaaatggcccgcctggctgaccgcccaacgacccccgcccattgacgtcaataatgacgtatgttcccatagtaacgccaatagggactttccattgacgtcaatgggtggagtatttacggtaaactgcccacttggcagtacatcaagtgtatcatatgccaagtacgccccctattgacgtcaatgacggtaaatggcccgcctggcattatgcccagtacatgaccttatgggactttcctacttggcagtacatctacgtattagtcatcgctattaccatggtgatgcggttttggcagtacatcaatgggcgtggatagcggtttgactcacggggatttccaagtctccaccccattgacgtcaatgggagtttgttttggcaccaaaatcaacgggactttccaaaatgtcgtaacaactccgccccattgacgcaaatgggcggtaggcgtgtacggtgggaggtctatataagcagagctcgtttagtgaaccgtcagatcgcctggagacgccatccacgctgttttgacctccatagaagacaccgggaccgatccagcctccggtcgaccgatcctgagaacttcagggtgagtttggggacccttgattgttctttctttttcgctattgtaaaattcatgttatatggagggggcaaagttttcagggtgttgtttagaatgggaagatgtcccttgtatcaccatggaccctcatgataattttgtttctttcactttctactctgttgacaaccattgtctcctcttattttcttttcattttcttgtaactttttcgttaaactttagcttgcatttgtaacgaatttttaaattcacttttgtttatttgtcagattgtaagtactttctctaatcacttttttttcaaggcaatcagggtatattatattgtacttcagcacagttttagagaacaattgttataattaaatgataaggtagaatatttctgcatataaattctggctggcgtggaaatattcttattggtagaaacaactacatcctggtcatcatcctgcctttctctttatggttacaatgatatacactgtttgagatgaggataaaatactctgagtccaaaccgggcccctctgctaaccatgttcatgccttcttctttttcctacagctcctgggcaacgtgctggttattgtgctgtctcatcattttggcaaagaattcctcgagatgggtgcgagagcgtcggtattaagcgggggagaattagataaatgggaaaaaattcggttaaggccagggggaaagaaacaatataaactaaaacatatagtatgggcaagcagggagctagaacgattcgcagttaatcctggccttttagagacatcagaaggctgtagacaaatactgggacagctacaaccatcccttcagacaggatcagaagaacttagatcattatataatacaatagcagtcctctattgtgtgcatcaaaggatagatgtaaaagacaccaaggaagccttagataagatagaggaagagcaaaacaaaagtaagaaaaaggcacagcaagcagcagctgacacaggaaacaacagccaggtcagccaaaattaccctatagtgcagaacctccaggggcaaatggtacatcaggccatatcacctagaactttaaatgcatgggtaaaagtagtagaagagaaggctttcagcccagaagtaatacccatgttttcagcattatcagaaggagccaccccacaagatttaaataccatgctaaacacagtggggggacatcaagcagccatgcaaatgttaaaagagaccatcaatgaggaagctgcagaatgggatagattgcatccagtgcatgcagggcctattgcaccaggccagatgagagaaccaaggggaagtgacatagcaggaactactagtacccttcaggaacaaataggatggatgacacataatccacctatcccagtaggagaaatctataaaagatggataatcctgggattaaataaaatagtaagaatgtatagccctaccagcattctggacataagacaaggaccaaaggaaccctttagagactatgtagaccgattctataaaactctaagagccgagcaagcttcacaagaggtaaaaaattggatgacagaaaccttgttggtccaaaatgcgaacccagattgtaagactattttaaaagcattgggaccaggagcgacactagaagaaatgatgacagcatgtcagggagtggggggacccggccataaagcaagagttttggctgaagcaatgagccaagtaacaaatccagctaccataatgatacagaaaggcaattttaggaaccaaagaaagactgttaagtgtttcaattgtggcaaagaagggcacatagccaaaaattgcagggcccctaggaaaaagggctgttggaaatgtggaaaggaaggacaccaaatgaaagattgtactgagagacaggctaattttttagggaagatctggccttcccacaagggaaggccagggaattttcttcagagcagaccagagccaacagccccaccagaagagagcttcaggtttggggaagagacaacaactccctctcagaagcaggagccgatagacaaggaactgtatcctttagcttccctcagatcactctttggcagcgacccctcgtcacaaccggggaccacgaccccaggcaaagcaagagttttggctgaagcaatgagcaccggtgattacaaagacgatgacgataagatggccccaaagaagaagcggaaggtcggtatccacggagtcccagcagccgacaagaagtacagcatcggcctggacatcggcaccaactctgtgggctgggccgtgatcaccgacgagtacaaggtgcccagcaagaaattcaaggtgctgggcaacaccgaccggcacagcatcaagaagaacctgatcggagccctgctgttcgacagcggcgaaacagccgaggccacccggctgaagagaaccgccagaagaagatacaccagacggaagaaccggatctgctatctgcaagagatcttcagcaacgagatggccaaggtggacgacagcttcttccacagactggaagagtccttcctggtggaagaggataagaagcacgagcggcaccccatcttcggcaacatcgtggacgaggtggcctaccacgagaagtaccccaccatctaccacctgagaaagaaactggtggacagcaccgacaaggccgacctgcggctgatctatctggccctggcccacatgatcaagttccggggccacttcctgatcgagggcgacctgaaccccgacaacagcgacgtggacaagctgttcatccagctggtgcagacctacaaccagctgttcgaggaaaaccccatcaacgccagcggcgtggacgccaaggccatcctgtctgccagactgagcaagagcagacggctggaaaatctgatcgcccagctgcccggcgagaagaagaatggcctgttcggcaacctgattgccctgagcctgggcctgacccccaacttcaagagcaacttcgacctggccgaggatgccaaactgcagctgagcaaggacacctacgacgacgacctggacaacctgctggcccagatcggcgaccagtacgccgacctgtttctggccgccaagaacctgtccgacgccatcctgctgagcgacatcctgagagtgaacaccgagatcaccaaggcccccctgagcgcctctatgatcaagagatacgacgagcaccaccaggacctgaccctgctgaaagctctcgtgcggcagcagctgcctgagaagtacaaagagattttcttcgaccagagcaagaacggctacgccggctacattgacggcggagccagccaggaagagttctacaagttcatcaagcccatcctggaaaagatggacggcaccgaggaactgctcgtgaagctgaacagagaggacctgctgcggaagcagcggaccttcgacaacggcagcatcccccaccagatccacctgggagagctgcacgccattctgcggcggcaggaagatttttacccattcctgaaggacaaccgggaaaagatcgagaagatcctgaccttccgcatcccctactacgtgggccctctggccaggggaaacagcagattcgcctggatgaccagaaagagcgaggaaaccatcaccccctggaacttcgaggaagtggtggacaagggcgcttccgcccagagcttcatcgagcggatgaccaacttcgataagaacctgcccaacgagaaggtgctgcccaagcacagcctgctgtacgagtacttcaccgtgtataacgagctgaccaaagtgaaatacgtgaccgagggaatgagaaagcccgccttcctgagcggcgagcagaaaaaggccatcgtggacctgctgttcaagaccaaccggaaagtgaccgtgaagcagctgaaagaggactacttcaagaaaatcgagtgcttcgactccgtggaaatctccggcgtggaagatcggttcaacgcctccctgggcacataccacgatctgctgaaaattatcaaggacaaggacttcctggacaatgaggaaaacgaggacattctggaagatatcgtgctgaccctgacactgtttgaggacagagagatgatcgaggaacggctgaaaacctatgcccacctgttcgacgacaaagtgatgaagcagctgaagcggcggagatacaccggctggggcaggctgagccggaagctgatcaacggcatccgggacaagcagtccggcaagacaatcctggatttcctgaagtccgacggcttcgccaacagaaacttcatgcagctgatccacgacgacagcctgacctttaaagaggacatccagaaagcccaggtgtccggccagggcgatagcctgcacgagcacattgccaatctggccggcagccccgccattaagaagggcatcctgcagacagtgaaggtggtggacgagctcgtgaaagtgatgggccggcacaagcccgagaacatcgtgatcgaaatggccagagagaaccagaccacccagaagggacagaagaacagccgcgagagaatgaagcggatcgaagagggcatcaaagagctgggcagccagatcctgaaagaacaccccgtggaaaacacccagctgcagaacgagaagctgtacctgtactacctgcagaatgggcgggatatgtacgtggaccaggaactggacatcaaccggctgtccgactacgatgtggaccatatcgtgcctcagagctttctgaaggacgactccatcgacaacaaggtgctgaccagaagcgacaagaaccggggcaagagcgacaacgtgccctccgaagaggtcgtgaagaagatgaagaactactggcggcagctgctgaacgccaagctgattacccagagaaagttcgacaatctgaccaaggccgagagaggcggcctgagcgaactggataaggccggcttcatcaagagacagctggtggaaacccggcagatcacaaagcacgtggcacagatcctggactcccggatgaacactaagtacgacgagaatgacaagctgatccgggaagtgaaagtgatcaccctgaagtccaagctggtgtccgatttccggaaggatttccagttttacaaagtgcgcgagatcaacaactaccaccacgcccacgacgcctacctgaacgccgtcgtgggaaccgccctgatcaaaaagtaccctaagctggaaagcgagttcgtgtacggcgactacaaggtgtacgacgtgcggaagatgatcgccaagagcgagcaggaaatcggcaaggctaccgccaagtacttcttctacagcaacatcatgaactttttcaagaccgagattaccctggccaacggcgagatccggaagcggcctctgatcgagacaaacggcgaaaccggggagatcgtgtgggataagggccgggattttgccaccgtgcggaaagtgctgagcatgccccaagtgaatatcgtgaaaaagaccgaggtgcagacaggcggcttcagcaaagagtctatcctgcccaagaggaacagcgataagctgatcgccagaaagaaggactgggaccctaagaagtacggcggcttcgacagccccaccgtggcctattctgtgctggtggtggccaaagtggaaaagggcaagtccaagaaactgaagagtgtgaaagagctgctggggatcaccatcatggaaagaagcagcttcgagaagaatcccatcgactttctggaagccaagggctacaaagaagtgaaaaaggacctgatcatcaagctgcctaagtactccctgttcgagctggaaaacggccggaagagaatgctggcctctgccggcgaactgcagaagggaaacgaactggccctgccctccaaatatgtgaacttcctgtacctggccagccactatgagaagctgaagggctcccccgaggataatgagcagaaacagctgtttgtggaacagcacaagcactacctggacgagatcatcgagcagatcagcgagttctccaagagagtgatcctggccgacgctaatctggacaaagtgctgtccgcctacaacaagcaccgggataagcccatcagagagcaggccgagaatatcatccacctgtttaccctgaccaatctgggagcccctgccgccttcaagtactttgacaccaccatcgaccggaagaggtacaccagcaccaaagaggtgctggacgccaccctgatccaccagagcatcaccggcctgtacgagacacggatcgacctgtctcagctgggaggcgacaagcgtcctgctgctactaagaaagctggtcaagctaagaaaaagaaagctagagcttgatatcctgcagacgcgtaggatccgtcgaggaattcactcctcaggtgcaggctgcctatcagaaggtggtggctggtgtggccaatgccctggctcacaaataccactgagatctttttccctctgccaaaaattatggggacatcatgaagccccttgagcatctgacttctggctaataaaggaaatttattttcattgcaatagtgtgttggaattttttgtgtctctcactcggaaggacatatgggagggcaaatcatttaaaacatcagaatgagtatttggtttagagtttggcaacatatgcccatatgctggctgccatgaacaaaggttggctataaagaggtcatcagtatatgaaacagccccctgctgtccattccttattccatagaaaagccttgacttgaggttagattttttttatattttgttttgtgttatttttttctttaacatccctaaaattttccttacatgttttactagccagatttttcctcctctcctgactactcccagtcatagctgtccctcttctcttatggagatccctcgacggatcggccgcaattcgtaatcatgtcatagctgtttcctgtgtgaaattgttatccgctcacaattccacacaacatacgagccggaagcataaagtgtaaagcctggggtgcctaatgagtgagctaactcacattaattgcgttgcgctcactgcccgctttccagtcgggaaacctgtcgtgccagctgcattaatgaatcggccaacgcgcggggagaggcggtttgcgtattgggcgctcttccgcttcctcgctcactgactcgctgcgctcggtcgttcggctgcggcgagcggtatcagctcactcaaaggcggtaatacggttatccacagaatcaggggataacgcaggaaagaacatgtgagcaaaaggccagcaaaaggccaggaaccgtaaaaaggccgcgttgctggcgtttttccataggctccgcccccctgacgagcatcacaaaaatcgacgctcaagtcagaggtggcgaaacccgacaggactataaagataccaggcgtttccccctggaagctccctcgtgcgctctcctgttccgaccctgccgcttaccggatacctgtccgcctttctcccttcgggaagcgtggcgctttctcatagctcacgctgtaggtatctcagttcggtgtaggtcgttcgctccaagctgggctgtgtgcacgaaccccccgttcagcccgaccgctgcgccttatccggtaactatcgtcttgagtccaacccggtaagacacgacttatcgccactggcagcagccactggtaacaggattagcagagcgaggtatgtaggcggtgctacagagttcttgaagtggtggcctaactacggctacactagaagaacagtatttggtatctgcgctctgctgaagccagttaccttcggaaaaagagttggtagctcttgatccggcaaacaaaccaccgctggtagcggtggtttttttgtttgcaagcagcagattacgcgcagaaaaaaaggatctcaagaagatcctttgatcttttctacggggtctgacgctcagtggaacgaaaactcacgttaagggattttggtcatgagattatcaaaaaggatcttcacctagatccttttaaattaaaaatgaagttttaaatcaatctaaagtatatatgagtaaacttggtctgacagttaccaatgcttaatcagtgaggcacctatctcagcgatctgtctatttcgttcatccatagttgcctgactccccgtcgtgtagataactacgatacgggagggcttaccatctggccccagtgctgcaatgataccgcgagacccacgctcaccggctccagatttatcagcaataaaccagccagccggaagggccgagcgcagaagtggtcctgcaactttatccgcctccatccagtctattaattgttgccgggaagctagagtaagtagttcgccagttaatagtttgcgcaacgttgttgccattgctacaggcatcgtggtgtcacgctcgtcgtttggtatggcttcattcagctccggttcccaacgatcaaggcgagttacatgatcccccatgttgtgcaaaaaagcgggttagctccttcggtcctccgatcgttgtcagaagtaagttggccgcagtgttatcactcatggttatggcagcactgcataattctcttactgtcatgccatccgtaagatgcttttctgtgactggtgagtactcaaccaagtcattctgagaatagtgtatgcggcgaccgagttgctcttgcccggcgtcaatacgggataataccgcgccacatagcagaactttaaaagtgctcatcattggaaaacgttcttcggggcgaaaactctcaaggatcttaccgctgttgagatccagttcgatgtaacccactcgtgcacccaactgatcttcagcatcttttactttcaccagcgtttctgggtgagcaaaaacaggaaggcaaaatgccgcaaaaaagggaataagggcgacacggaaatgttgaatactcatactcttcctttttcaatattattgaagcatttatcagggttattgtctcatgagcggatacatatttgaatgtatttagaaaaataaacaaataggggttccgcgcacatttccccgaaaagtgccacctaaattgtaagcgttaatattttgttaaaattcgcgttaaatttttgttaaatcagctcattttttaaccaataggccgaaatcggcaaaatcccttataaatcaaaagaatagaccgagatagggttgagtgttgttccagtttggaacaagagtccactattaaagaacgtggactccaacgtcaaagggcgaaaaaccgtctatcagggcgatggcccactacgtgaaccatcaccctaatcaagttttttggggtcgaggtgccgtaaagcactaaatcggaaccctaaagggagcccccgatttagagcttgacggggaaagccggcgaacgtggcgagaaaggaagggaagaaagcgaaaggagcgggcgctagggcgctggcaagtgtagcggtcacgctgcgcgtaaccaccacacccgccgcgcttaatgcgccgctacagggcgcgtcccattcgccattcaggctgcgcaactgttgggaagggcgatcggtgcgggcctcttcgctattacgccagctggcgaaagggggatgtgctgcaaggcgattaagttgggtaacgccagggttttcccagtcacgacgttgtaaaacgacggccagtgagcgcgcgtaatacgactcactatagggcgaattggagctccaccgcggtg

SEQ ID NO: 35 - DNA, 20 bp, Artificial Sequence
  GFP target sequence
  GFP target sequence
cgaggagctgttcaccgggg

SEQ ID NO: 36 - DNA, 27 bp, Artificial Sequence
  primer
attgcggaagttcctcttcttaccctg

SEQ ID NO: 37 - DNA, 27 bp, Artificial Sequence
  primer
ttcctgggaagggtggattatgacggg

SEQ ID NO: 38 - DNA, 20 bp, Artificial Sequence
  target sequence
cgaggagctgttcaccgggg

SEQ ID NO: 39 - DNA, 23 bp, Artificial Sequence
  primer
tctgagtggcaaaggaccttagg

SEQ ID NO: 40 - DNA, 26 bp, Artificial Sequence
  primer
gaagtcgtgctgcttcatgtggtcgg